European Patent Application EP 4 151 233 A1, published March 22, 2023. Title: FORMULATION COMPRISING ANTI-IL-23P19 ANTIBODY, METHOD FOR PREPARING SAME AND USE THEREOF. Applicant: Innovent Biologics (Suzhou) Co., Ltd. The sequence listing filed with the application follows.

SEQUENCE LISTING (10 sequences)

SEQ ID NO: 1 - protein, 10 aa, Artificial Sequence
  VH CDR1
GYTFTSYLMH

SEQ ID NO: 2 - protein, 10 aa, Artificial Sequence
  VH CDR2
YINPYNEGTN

SEQ ID NO: 3 - protein, 6 aa, Artificial Sequence
  VH CDR3
NWDLPY

SEQ ID NO: 4 - protein, 11 aa, Artificial Sequence
  VL CDR1
RASQSISDYLH

SEQ ID NO: 5 - protein, 7 aa, Artificial Sequence
  VL CDR2
YASQSMS

SEQ ID NO: 6 - protein, 9 aa, Artificial Sequence
  VL CDR3
QQGHSFPFT

SEQ ID NO: 7 - protein, 115 aa, Artificial Sequence
  VH
QVQLVQSGAEVKKPGASVKVSCKASGYTFTSYLMHWVRQAPGQGLEWMGYINPYNEGTNYAQKFQGRVTMTRDTSISTAYMELSRLRSDDTAVYYCARNWDLPYWGQGTLVTVSS

SEQ ID NO: 8 - protein, 107 aa, Artificial Sequence
  VL
DIQMTQSPSSLSASVGDRVTITCRASQSISDYLHWYQQKPGKAPKLLIKYASQSMSGVPSRFSGSGSGSDFTLTISSLQPEDFATYYCQQGHSFPFTFGQGTKLEIK

SEQ ID NO: 9 - protein, 444 aa, Artificial Sequence
  HC
QVQLVQSGAEVKKPGASVKVSCKASGYTFTSYLMHWVRQAPGQGLEWMGYINPYNEGTNYAQKFQGRVTMTRDTSISTAYMELSRLRSDDTAVYYCARNWDLPYWGQGTLVTVSSASTKGPSVFPLAPSSKSTSGGTAALGCLVKDYFPEPVTVSWNSGALTSGVHTFPAVLQSSGLYSLSSVVTVPSSSLGTQTYICNVNHKPSNTKVDKKVEPKSCDKTHTCPPCPAPELLGGPSVFLFPPKPKDTLYITREPEVTCVVVDVSHEDPEVKFNWYVDGVEVHNAKTKPREEQYNSTYRVVSVLTVLHQDWLNGKEYKCKVSNKALPAPIEKTISKAKGQPREPQVYTLPPSRDELTKNQVSLTCLVKGFYPSDIAVEWESNGQPENNYKTTPPVLDSDGSFFLYSKLTVDKSRWQQGNVFSCSVMHEALHNHYTQKSLSLSPG

SEQ ID NO: 10 - protein, 214 aa, Artificial Sequence
  LC
DIQMTQSPSSLSASVGDRVTITCRASQSISDYLHWYQQKPGKAPKLLIKYASQSMSGVPSRFSGSGSGSDFTLTISSLQPEDFATYYCQQGHSFPFTFGQGTKLEIKRTVAAPSVFIFPPSDEQLKSGTASVVCLLNNFYPREAKVQWKVDNALQSGNSQESVTEQDSKDSTYSLSSTLTLSKADYEKHKVYACEVTHQGLSSPVTKSFNRGEC